European Patent Application EP 4 410 839 A1, published August 7, 2024. Title: ANTI-B7-H3 ANTIBODY AND APPLICATION THEREOF. Applicant: Bio-Thera Solutions, Ltd. The sequence listing filed with the application follows.

SEQUENCE LISTING (52 sequences)

SEQ ID NO: 1 - protein, 688 aa, synthetic construct
MLRRRGSPGMGVHVGAALGALWFCLTGALEVQVPEDPVVALVGTDATLCCSFSPEPGFSLAQLNLIWQLTDTKQLVHSFAEGQDQGSAYANRTALFPDLLAQGNASLRLQRVRVADEGSFTCFVSIRDFGSAAVSLQVAAPYSKPSMTLEPNKDLRPGDTVTITCSSYQGYPEAEVFWQDGQGVPLTGNVTTSQMANEQGLFDVHSILRVVLGANGTYSCLVRNPVLQQDAHSSVTITPQRSPTGAVEVQVPEDPVVALVGTDATLRCSFSPEPGFSLAQLNLIWQLTDTKQLVHSFTEGRDQGSAYANRTALFPDLLAQGNASLRLQRVRVADEGSFTCFVSIRDFGSAAVSLQVAAPYSKPSMTLEPNKDLRPGDTVTITCSSYRGYPEAEVFWQDGQGVPLTGNVTTSQMANEQGLFDVHSVLRVVLGANGTYSCLVRNPVLQQDAHGSVTITGQPMTDKTHTCPPCPAPELLGGPSVFLFPPKPKDTLMISRTPEVTCVVVDVSHEDPEVKFNWYVDGVEVHNAKTKPREEQYNSTYRVVSVLTVLHQDWLNGKEYKCKVSNKALPAPIEKTISKAKGQPREPQVYTLPPSRDELTKNQVSLTCLVKGFYPSDIAVEWESNGQPENNYKTTPPVLDSDGSFFLYSKLTVDKSRWQQGNVFSCSVMHEALHNHYTQKSLSLSPGK

SEQ ID NO: 2 - protein, 461 aa, Homo sapiens
MLRRRGSPGMGVHVGAALGALWFCLTGALEVQVPEDPVVALVGTDATLCCSFSPEPGFSLAQLNLIWQLTDTKQLVHSFAEGQDQGSAYANRTALFPDLLAQGNASLRLQRVRVADEGSFTCFVSIRDFGSAAVSLQVAAPYSKPSMTLEPNKDLRPGDTVTITCSSYQGYPEAEVFWQDGQGVPLTGNVTTSQMANEQGLFDVHSILRVVLGANGTYSCLVRNPVLQQDAHSSVTITPQRSPTGAVEVQVPEDPVVALVGTDATLRCSFSPEPGFSLAQLNLIWQLTDTKQLVHSFTEGRDQGSAYANRTALFPDLLAQGNASLRLQRVRVADEGSFTCFVSIRDFGSAAVSLQVAAPYSKPSMTLEPNKDLRPGDTVTITCSSYRGYPEAEVFWQDGQGVPLTGNVTTSQMANEQGLFDVHSVLRVVLGANGTYSCLVRNPVLQQDAHGSVTITGQPMT

SEQ ID NO: 3 - protein, 227 aa, Homo sapiens
DKTHTCPPCPAPELLGGPSVFLFPPKPKDTLMISRTPEVTCVVVDVSHEDPEVKFNWYVDGVEVHNAKTKPREEQYNSTYRVVSVLTVLHQDWLNGKEYKCKVSNKALPAPIEKTISKAKGQPREPQVYTLPPSRDELTKNQVSLTCLVKGFYPSDIAVEWESNGQPENNYKTTPPVLDSDGSFFLYSKLTVDKSRWQQGNVFSCSVMHEALHNHYTQKSLSLSPGK

SEQ ID NO: 4 - protein, 471 aa, synthetic construct
MLRRRGSPGMGVHVGAALGALWFCLTGALEVQVPEDPVVALVGTDATLCCSFSPEPGFSLAQLNLIWQLTDTKQLVHSFAEGQDQGSAYANRTALFPDLLAQGNASLRLQRVRVADEGSFTCFVSIRDFGSAAVSLQVAAPYSKPSMTLEPNKDLRPGDTVTITCSSYQGYPEAEVFWQDGQGVPLTGNVTTSQMANEQGLFDVHSILRVVLGANGTYSCLVRNPVLQQDAHSSVTITPQRSPTGAVEVQVPEDPVVALVGTDATLRCSFSPEPGFSLAQLNLIWQLTDTKQLVHSFTEGRDQGSAYANRTALFPDLLAQGNASLRLQRVRVADEGSFTCFVSIRDFGSAAVSLQVAAPYSKPSMTLEPNKDLRPGDTVTITCSSYRGYPEAEVFWQDGQGVPLTGNVTTSQMANEQGLFDVHSVLRVVLGANGTYSCLVRNPVLQQDAHGSVTITGQPMTHHHHHHHHHH

SEQ ID NO: 5 - protein, 10 aa, synthetic construct
HHHHHHHHHH

SEQ ID NO: 6 - protein, 5 aa, synthetic construct
DYDIN

SEQ ID NO: 7 - protein, 17 aa, synthetic construct
WIFPGDDTTKYNEKFKG

SEQ ID NO: 8 - protein, 6 aa, synthetic construct
SPSFDY

SEQ ID NO: 9 - protein, 10 aa, synthetic construct
SASSTIGFMY

SEQ ID NO: 10 - protein, 11 aa, synthetic construct
KASQDINRFLS

SEQ ID NO: 11 - protein, 15 aa, synthetic construct
RASKSVSTSGYSYMH

SEQ ID NO: 12 - protein, 11 aa, synthetic construct
RATGNIHNYLA

SEQ ID NO: 13 - protein, 11 aa, synthetic construct
RASKNIYSFLG

SEQ ID NO: 14 - protein, 7 aa, synthetic construct
DTSKLAS

SEQ ID NO: 15 - protein, 7 aa, synthetic construct
RANRLRD

SEQ ID NO: 16 - protein, 7 aa, synthetic construct
LVSNLES

SEQ ID NO: 17 - protein, 7 aa, synthetic construct
SAKTLAD

SEQ ID NO: 18 - protein, 7 aa, synthetic construct
NAKTLAE

SEQ ID NO: 19 - protein, 8 aa, synthetic construct
HQRSSYPT

SEQ ID NO: 20 - protein, 10 aa, synthetic construct
LQYDEFPPFT

SEQ ID NO: 21 - protein, 7 aa, synthetic construct
QHIRELT

SEQ ID NO: 22 - protein, 9 aa, synthetic construct
QHFWSIPWT

SEQ ID NO: 23 - protein, 10 aa, synthetic construct
QHHYGTPPYT

SEQ ID NO: 24 - protein, 115 aa, synthetic construct
QVQLQQSGPELVKPGASVRISCKASGYTFTDYDINWVQQRPGQGLEWIGWIFPGDDTTKYNEKFKGRATLTADKSSNTAYMQLNGLTSENSAVYFCARSPSFDYWGQGTLVTVSS

SEQ ID NO: 25 - protein, 105 aa, synthetic construct
QIVLTQSPAIMSASPGERVTMTCSASSTIGFMYWYQQKPGTSPKRWIYDTSKLASGVPARFSVSGSGTSYSLTISSMEAEDAATYYCHQRSSYPTFGGGTKLEIK

SEQ ID NO: 26 - protein, 108 aa, synthetic construct
DIKMTQSPSSMYASLGERVTITCKASQDINRFLSWFQQKPGKSPKTLIYRANRLRDGVPSRFSGNGSGQDYSLTISSLEYEDMGIYYCLQYDEFPPFTFGSGTKLEIK

SEQ ID NO: 27 - protein, 109 aa, synthetic construct
DIVLTQSPASLAVSLGQRATISCRASKSVSTSGYSYMHWNQQKPGQPPRLLIYLVSNLESGVPARFSGSGSGTDFTLNIHPVEEEDAATYYCQHIRELTFGAGTKLELK

SEQ ID NO: 28 - protein, 107 aa, synthetic construct
DIQMTQSTASLSAFVGETVTITCRATGNIHNYLAWYHQKQGKSPHLLVYSAKTLADGVPSRFSGSGSGTQYSLQINSLHPEDFGTYYCQHFWSIPWTFGGGTKLEIK

SEQ ID NO: 29 - protein, 108 aa, synthetic construct
DIQMTQSPASLSASVGETVTITCRASKNIYSFLGWIQQRQGKSPQSLVYNAKTLAEGVPSRFSGSGSGTQFSLKINSLQPEDFGNYYCQHHYGTPPYTFGGGTKLEIK

SEQ ID NO: 30 - protein, 452 aa, synthetic construct
QVQLVQSGAEVKKPGSSVKVSCKASGYTFTNYVMHWVRQAPGQGLEWMGYINPYNDDVKYNEKFKGRVTITADESTSTAYMELSSLRSEDTAVYYCARWGYYGSPLYYFDYWGQGTLVTVSSASTKGPSVFPLAPSSKSTSGGTAALGCLVKDYFPEPVTVSWNSGALTSGVHTFPAVLQSSGLYSLSSVVTVPSSSLGTQTYICNVNHKPSNTKVDKRVEPKSCDKTHTCPPCPAPELLGGPSVFLFPPKPKDTLMISRTPEVTCVVVDVSHEDPEVKFNWYVDGVEVHNAKTKPREEQYNSTYRVVSVLTVLHQDWLNGKEYKCKVSNKALPAPIEKTISKAKGQPREPQVYTLPPSREEMTKNQVSLTCLVKGFYPSDIAVEWESNGQPENNYKTTPPVLDSDGSFFLYSKLTVDKSRWQQGNVFSCSVMHEALHNHYTQKSLSLSPGK

SEQ ID NO: 31 - protein, 213 aa, synthetic construct
EIVLTQSPATLSLSPGERATLSCRASSRLIYMHWYQQKPGQAPRPLIYATSNLASGIPARFSGSGSGTDFTLTISSLEPEDFAVYYCQQWNSNPPTFGQGTKVEIKRTVAAPSVFIFPPSDEQLKSGTASVVCLLNNFYPREAKVQWKVDNALQSGNSQESVTEQDSKDSTYSLSSTLTLSKADYEKHKVYACEVTHQGLSSPVTKSFNRGEC

SEQ ID NO: 32 - protein, 330 aa, synthetic construct [sequence omitted]

SEQ ID NO: 33 - protein, 327 aa, synthetic construct
ASTKGPSVFPLAPCSRSTSESTAALGCLVKDYFPEPVTVSWNSGALTSGVHTFPAVLQSSGLYSLSSVVTVPSSSLGTKTYTCNVDHKPSNTKVDKRVESKYGPPCPPCPAPEFLGGPSVFLFPPKPKDTLMISRTPEVTCVVVDVSQEDPEVQFNWYVDGVEVHNAKTKPREEQFNSTYRVVSVLTVLHQDWLNGKEYKCKVSNKGLPSSIEKTISKAKGQPREPQVYTLPPSQEEMTKNQVSLTCLVKGFYPSDIAVEWESNGQPENNYKTTPPVLDSDGSFFLYSRLTVDKSRWQEGNVFSCSVMHEALHNHYTQKSLSLSLGK

SEQ ID NO: 34 - protein, 107 aa, synthetic construct [sequence omitted]

SEQ ID NO: 35 - protein, 115 aa, synthetic construct
EVQLVQSGAEVKKSGESLKISCKASGYTFTDYDINWVRQMPGKGLEWMGWIFPGDDTTKYNEKFKGQVTISADKSTNTAYLQWSSLKASDTAMYYCARSPSFDYWGQGTLVTVSS

SEQ ID NO: 36 - protein, 115 aa, synthetic construct
EVQLVQSGAEVKKSGESLKISCKASGYTFTDYDINWVRQMPGKGLEWIGWIFPGDDTTKYNEKFKGQVTLSADKSTNTAYMQWSSLKASDTAMYYCARSPSFDYWGQGTLVTVSS

SEQ ID NO: 37 - protein, 115 aa, synthetic construct
EVQLVESGGGLVQPGGSLRLSCAASGYTFTDYDINWVRQAPGKGLEWVGWIFPGDDTTKYNEKFKGRFTISADKSKNTAYLQMNSLRAEDTAVYYCARSPSFDYWGQGTLVTVSS

SEQ ID NO: 38 - protein, 115 aa, synthetic construct
QVQLVQSGAEVKKPGASVKVSCKASGYTFTDYDINWVRQAPGQRLEWIGWIFPGDDTTKYNEKFKGRATLTADKSASTAYMELSSLRSEDTAVYYCARSPSFDYWGQGTLVTVSS

SEQ ID NO: 39 - protein, 105 aa, synthetic construct
QIVLTQSPGTLSLSPGERATLSCSASSTIGFMYWYQQKPGQAPRRWIYDTSKLASGVPDRFSVSGSGTDYTLTISRLEPEDFAVYYCHQRSSYPTFGQGTKVEIK

SEQ ID NO: 40 - protein, 105 aa, synthetic construct
QIVLTQSPGTLSLSPGERATLSCSASSTIGFMYWYQQKPGQAPRRWIYDTSKLASGVPDRFSGSGSGTDYTLTISRLEPEDFAVYYCHQRSSYPTFGQGTKVEIK

SEQ ID NO: 41 - protein, 105 aa, synthetic construct
QIVLTQSPSSLSASVGDRVTITCSASSTIGFMYWYQQKPGKAPKRWIYDTSKLASGVPSRFSVSGSGTDYTLTISSLQPEDFATYYCHQRSSYPTFGQGTKVEIK

SEQ ID NO: 42 - protein, 451 aa, synthetic construct
QVQLQQSGSELKKPGASVKVSCKASGYTFTNYGMNWVKQAPGQGLKWMGWINTYTGEPTYTDDFKGRFAFSLDTSVSTAYLQISSLKADDTAVYFCARGGFGSSYWYFDVWGQGTLVTVSSASTKGPSVFPLAPSSKSTSGGTAALGCLVKDYFPEPVTVSWNSGALTSGVHTFPAVLQSSGLYSLSSVVTVPSSSLGTQTYICNVNHKPSNTKVDKKVEPKSCDKTHTCPPCPAPELLGGPSVFLFPPKPKDTLMISRTPEVTCVVVDVSHEDPEVKFNWYVDGVEVHNAKTKPREEQYNSTYRVVSVLTVLHQDWLNGKEYKCKVSNKALPAPIEKTISKAKGQPREPQVYTLPPSRDELTKNQVSLTCLVKGFYPSDIAVEWESNGQPENNYKTTPPVLDSDGSFFLYSKLTVDKSRWQQGNVFSCSVMHEALHNHYTQKSLSLSPGK

SEQ ID NO: 43 - protein, 214 aa, synthetic construct
DIQLTQSPSSLSASVGDRVSITCKASQDVSIAVAWYQQKPGKAPKLLIYSASYRYTGVPDRFSGSGSGTDFTLTISSLQPEDFAVYYCQQHYITPLTFGAGTKVEIKRTVAAPSVFIFPPSDEQLKSGTASVVCLLNNFYPREAKVQWKVDNALQSGNSQESVTEQDSKDSTYSLSSTLTLSKADYEKHKVYACEVTHQGLSSPVTKSFNRGEC

SEQ ID NO: 44 - protein, 534 aa, Homo sapiens
MLRRRGSPGMGVHVGAALGALWFCLTGALEVQVPEDPVVALVGTDATLCCSFSPEPGFSLAQLNLIWQLTDTKQLVHSFAEGQDQGSAYANRTALFPDLLAQGNASLRLQRVRVADEGSFTCFVSIRDFGSAAVSLQVAAPYSKPSMTLEPNKDLRPGDTVTITCSSYQGYPEAEVFWQDGQGVPLTGNVTTSQMANEQGLFDVHSILRVVLGANGTYSCLVRNPVLQQDAHSSVTITPQRSPTGAVEVQVPEDPVVALVGTDATLRCSFSPEPGFSLAQLNLIWQLTDTKQLVHSFTEGRDQGSAYANRTALFPDLLAQGNASLRLQRVRVADEGSFTCFVSIRDFGSAAVSLQVAAPYSKPSMTLEPNKDLRPGDTVTITCSSYRGYPEAEVFWQDGQGVPLTGNVTTSQMANEQGLFDVHSVLRVVLGANGTYSCLVRNPVLQQDAHGSVTITGQPMTFPPEALWVTVGLSVCLIALLVALAFVCWRKIKQSCEEENAGAEDQDGEGEGSKTALQPLKHSDSKEDDGQEIA

SEQ ID NO: 45 - protein, 19 aa, synthetic construct
MEFGLSWVFLVAILKGVQC

SEQ ID NO: 46 - protein, 19 aa, synthetic construct
MKHLWFFLLLVAAPRWVLS

SEQ ID NO: 47 - protein, 22 aa, synthetic construct
MDMRVLAQLLGLLLLCFPGARC

SEQ ID NO: 48 - protein, 20 aa, synthetic construct
MVLQTQVFISLLLWISGAYG

SEQ ID NO: 49 - DNA, 1335 bp, synthetic construct
  source 1..1335: mol_type = other DNA
gaggtgcagctggtgcagagcggcgccgaggtgaagaagagcggcgagtccctgaagatctcctgtaaggctagcggctatacctttaccgattacgatatcaactgggtgcggcagatgcctggcaagggcctggagtggatcggctggatctttcccggcgatgacaccaccaagtacaacgagaagttcaagggccaggtgaccctgagcgctgataagtccaccaacaccgcctacatgcagtggtcctccctgaaggcctccgacaccgccatgtattattgcgcccggtcccccagcttcgactactggggccagggtaccctggttaccgttagcagcgcgagcaccaaaggcccgagcgtgtttccgctggccccgagcagcaaaagcaccagcggtggcaccgcagcgctgggttgcctggtgaaagattatttcccggaaccggtgacggtgtcgtggaactcaggcgccctgaccagcggcgtgcacaccttcccggctgtcctacagtcctcaggactctactccctcagcagcgtggtgaccgtgccctccagcagcttgggcacccagacctacatctgcaacgtgaatcacaagcccagcaacaccaaggtggacaagaaagttgagcccaaatcttgtgacaaaactcacacatgcccaccgtgcccagcacctgaactcctggggggaccgtcagtcttcctcttccccccaaaacccaaggacaccctcatgatctcccggacccctgaggtcacatgcgtggtggtggacgtgagccacgaagaccctgaggtcaagttcaactggtacgtggacggcgtggaggtgcataatgccaagacaaagccgcgggaggagcagtacaacagcacgtaccgtgtggtcagcgtcctcaccgtcctgcaccaggactggctgaatggcaaggagtacaagtgcaaggtctccaacaaagccctcccagcccccatcgagaaaaccatctccaaagccaaagggcagccccgagaaccacaggtgtacaccctgcccccatcccgggatgagctgaccaagaaccaggtcagcctgacctgcctggtcaaaggcttctatcccagcgacatcgccgtggagtgggagagcaatgggcagccggagaacaactacaagaccacgcctcccgtgctggactccgacggctccttcttcctctacagcaagctcaccgtggacaagagcaggtggcagcaggggaacgtcttctcatgctccgtgatgcatgaggctctgcacaaccactacacgcagaagagcctctccctgtctccgggtaaa

SEQ ID NO: 50 - protein, 445 aa, synthetic construct
EVQLVQSGAEVKKSGESLKISCKASGYTFTDYDINWVRQMPGKGLEWIGWIFPGDDTTKYNEKFKGQVTLSADKSTNTAYMQWSSLKASDTAMYYCARSPSFDYWGQGTLVTVSSASTKGPSVFPLAPSSKSTSGGTAALGCLVKDYFPEPVTVSWNSGALTSGVHTFPAVLQSSGLYSLSSVVTVPSSSLGTQTYICNVNHKPSNTKVDKKVEPKSCDKTHTCPPCPAPELLGGPSVFLFPPKPKDTLMISRTPEVTCVVVDVSHEDPEVKFNWYVDGVEVHNAKTKPREEQYNSTYRVVSVLTVLHQDWLNGKEYKCKVSNKALPAPIEKTISKAKGQPREPQVYTLPPSRDELTKNQVSLTCLVKGFYPSDIAVEWESNGQPENNYKTTPPVLDSDGSFFLYSKLTVDKSRWQQGNVFSCSVMHEALHNHYTQKSLSLSPGK

SEQ ID NO: 51 - DNA, 636 bp, synthetic construct
  source 1..636: mol_type = other DNA
cagatcgtgctgacccagagccccggcaccctgtccctgagccctggagagagggccaccctgagctgtagcgctagctccaccatcggctttatgtattggtatcagcagaagcctggccaggccccccggagatggatctacgacaccagcaagctggccagcggcgtgcctgacaggttttccggcagcggctccggcaccgactataccctgaccatcagcaggctggagcccgaggatttcgccgtgtattattgccaccagcggagcagctatcctacctttggccagggcaccaaggtggagatcaagcgtacggtggctgcaccatctgtcttcatcttcccgccatctgatgagcagttgaaatctggaactgcctctgttgtgtgcctgctgaataacttctatcccagagaggccaaagtacagtggaaggtggataacgccctccaatcgggtaactcccaggagagtgtcacagagcaggacagcaaggacagcacctacagcctcagcagcaccctgacgctgagcaaagcagactacgagaaacacaaagtctacgcctgcgaagtcacccatcagggcctgagctcgcccgtcacaaagagcttcaacaggggagagtgt

SEQ ID NO: 52 - protein, 212 aa, synthetic construct
QIVLTQSPGTLSLSPGERATLSCSASSTIGFMYWYQQKPGQAPRRWIYDTSKLASGVPDRFSGSGSGTDYTLTISRLEPEDFAVYYCHQRSSYPTFGQGTKVEIKRTVAAPSVFIFPPSDEQLKSGTASVVCLLNNFYPREAKVQWKVDNALQSGNSQESVTEQDSKDSTYSLSSTLTLSKADYEKHKVYACEVTHQGLSSPVTKSFNRGEC